European Patent Specification EP 3 090 048 B1, published February 15, 2023. Title: Maize Cytoplasmic Male Sterility (CMS) S-type Restorer Gene Rf3. Applicant: Dow AgroSciences, LLC Ren, Ruihua Nagel, Bruce Ye, Liang Gao, Yanxin Gibson, Ryan Paulraj, Sushmitha Mansfield, Tyler Mammadov, Jafar Kumpalta, Siva Thompson, Steve. The sequence listing filed with the application follows.

SEQUENCE LISTING (36 sequences)

SEQ ID NO: 1 - protein, 6 aa, zea mays
IVFFSS

SEQ ID NO: 2 - DNA, 15 bp, zea mays
attgttttcttcagt

SEQ ID NO: 3 - protein, 697 aa, zea mays
MDCCTRAHRPELALAFFGQLLRTGLRVDIIIANHLLKGFCEAKRTDEALDILLHRTPELGCVPDVFSYSILLKSLCDQGKSGQADDLLRMMAEGGAVCSPDVVAYNTVIDGFFKEGDVNKACDLFKEMVQRGIPPDFVTYSSVVHALCKARAMDKAEAFLRQMVNKGVLPNNWTYNNLIYGYSSTGQWKEAVRVFKEMRRHSILPDVVTLNMLMGSLCKYGKIKEARDVFDTMAMKGQNPDVFSYNIMLNGYATKGCLVDMTDLFDLMLGDGIAPVICTFNVLIKAYANCGMLDKAMIIFNEMRDHGVKPYVVTYTTVIAALCRIGKMDDAMEKFNQMIDQGVAPDKYAFHCLIQGFCTHGSLLKAKELILEIMNNGMRLDIVFFSSIINNLCKLGRVMEAQNIFDLTVNVGLHPTAVVYSMLMDGYCLVGKMEKALRVFDAMVSAGIEPYVVVYGTLVNGYCKIGRIDEGLSLFREMLQKGIKPSTILYNIIIDGLFQAGRTVPAKVKFHEMTESGIAINKCTYNIVLRGFFKNRCFDEAIFLFKELRAMNVKIDIITLNTMIAGMFQTRRVEEAKDLFASISRSGLVPCVVTYSIMITNLIKEGLVEEAEDMFSSMQNAGCEPNSRLLNHVVRELLKKNEIVRAGAYLSKIDERNFSLEHLTTMLLVDLFSSKGTCREHIRFLPAKYHFLAEASP

SEQ ID NO: 4 - DNA, 2094 bp, zea mays
atggactgctgcacccgcgcgcaccgcccagagctagcgctggccttcttcggccagctcctcaggacaggcttgcgcgtcgatatcatcatcgctaaccaccttctcaagggcttttgtgaagcgaagcggacagacgaggctttggacatccttctccacagaacgcctgagttgggctgtgtgcccgatgttttctcgtacagcatacttctgaagagcctctgcgaccaaggaaagagtggccaggcagatgatttgctacggatgatggctgaagggggagctgtctgctcgcccgacgtggttgcctacaatacagtaatcgacggcttctttaaggagggtgacgtaaataaagcatgtgatctattcaaagaaatggtacagcggggcattccacctgattttgtgacttatagctctgtggttcatgccctgtgtaaggcaagagcaatggacaaggcagaggctttccttcgacaaatggtcaataaaggtgttctgccaaataactggacatataataacttgatatatggatactcctccacaggacagtggaaggaggcagttagggtatttaaagaaatgagaagacacagcatcttaccagatgttgttactttgaacatgttgatgggttccctttgcaagtatggaaaaatcaaggaagctagagatgtttttgacacaatggcaatgaagggccaaaatcctgatgttttctcgtacaatattatgctcaacgggtacgctactaaaggatgtctagttgatatgacagatctcttcgatttgatgctaggtgacggtattgcacctgtcatttgtacttttaatgtgctgatcaaggcatatgcaaactgtggaatgctagataaggctatgatcatcttcaatgaaatgagagaccatggagtgaaaccttatgtggtaacctatacgacagtgattgctgccctctgcagaatcggtaagatggatgatgctatggaaaaatttaatcagatgattgatcaaggagtagcacctgataaatatgcattccattgcctgattcaaggtttttgtactcatggtagtttactgaaagccaaggaattgattttggaaataatgaataatggcatgcgtcttgatattgttttcttcagttcgataattaacaacctttgcaaactgggaagggtaatggaggcacaaaatatatttgacttaactgtaaatgttggtctgcatcctactgctgtggtgtatagtatgcttatggatgggtactgtcttgttggcaagatggagaaagcattaagagtatttgatgctatggtgtcagctggcattgaaccatacgttgtagtgtatggtacacttgttaatggctattgtaaaattggaaggattgatgaaggattgagtcttttcagagaaatgctgcaaaagggaataaagccttcaactattttatacaacatcataattgatgggttatttcaggccgggagaacagttcctgcaaaggtgaaattccatgaaatgacagaaagtggtatcgctatcaacaaatgtacatacaacatagttcttcgtggattttttaaaaatagatgctttgatgaagcaatctttcttttcaaagaattacgtgcaatgaatgtaaagatcgatatcataactctcaataccatgatagctggaatgtttcaaaccaggagagttgaagaagctaaggatctgtttgcttctatctcgagaagtgggctggtgccttgtgttgtgacttacagtataatgatcacaaatcttataaaagaaggattggtggaagaggcagaagatatgttttcatccatgcagaatgctggctgtgagcccaattctcgattgctgaatcatgtagtcagggaattactaaagaaaaatgaaatagtcagggctggagcttacctgtccaagattgacgagaggaatttctcacttgaacatttaaccacaatgttgctggtcgatctcttctcaagcaaaggaacttgtagggaacacataagatttctccctgcaaagtatcattttcttgcagaggccagtccgtga

SEQ ID NO: 5 - protein, 5 aa, zea mays
IVLFS

SEQ ID NO: 6 - DNA, 15 bp, zea mays
attgttttattcagt

SEQ ID NO: 7 - protein, 814 aa, zea mays
MPSCARISSAVSTAAASSSSPPPHPPRCRRLAAATARVREGTLRPEEAHDLLDELQRRGTPVLERDLNGFLAAFARAPSSAACRSGPALAVALFNRAASRAQGPRVLSPTSHTYAILMDCCTRAHRPELALAFFGQLLRTGLRVDIIIANHLLKGFCEAKRTDEALDILLHRTPELGCVPDVFSYSILLKSLCDQGKSGQADDLLRMMSEGGAVCSPDVVAYNTVIDGFFKEGDVNKACDLFKEMVQRGIPPDFVTYSSVVHALCKARAMDKAEAFLRQMVNKGVLPNNWTYNNLIYGYSSTGQWKEAVRVFKEMRRHSILPDVVTFNMLMGSLCKYGKIKEARDVFDTMAMKGQNPDVFSYNIMLNGYATKGCLVDMTDLFDLMLGDGIAPVICTFNVLIKAYANCGMLDKAMIIFNEMRDHGVKPYVLTYTTVIAALCRIGKMDDAMEKFNQMIDQGVAPDKYAYHCLIQGFCTHGSLLKAKELISEIMNNGMHLDIVLFSSIINNLCKLGRVMDAQNIFDLTVNVGLHPTAVVYSMLMDGYCLVGKMENALRVFDAMVSAGIEPYDVVYGTLVNGYCKIGRIDEGLSLFREMLQNGIKPSTILYNIIIDGLFEAGRTVPAKVKFHEMTESGIAMYICTYIIVLRGLFKNRCFDEAIFLFKELRAMNVKIDIITLNTMIAGMFQTRRVEEAKDLFASISRSGLVPCVVTYSIMITNLIKEGLVEEAEDMFSSMQNAGCEPYSRLLNHVVRELLKKNEIVRAGAYLSKIDERNFSLEYLTTMLLVDLFSSKGTCREHIRFLPAKYHFLAEASP

SEQ ID NO: 8 - DNA, 2445 bp, zea mays
atgccgtcatgtgcccgcatctcctccgccgtctccaccgccgccgcatcctcctcctcgccgccgccgcatcctcctcgctgccgccgcctcgccgccgccacggcgcgcgtgcgggaggggacgctccgccctgaggaagcacacgacctgctcgacgagttgcagcgtcgaggcacgcccgttctcgagcgcgatctgaacggcttcctcgcggcgttcgcgcgtgcgccgtcctccgccgcctgcaggagtggccctgccctcgccgtcgcgctcttcaaccgcgcggcgtctcgggctcaaggaccgcgggtgctgtcccccacatcccacacctacgccatcctcatggactgctgcacccgcgcgcaccgcccagagctagcgctggcgttcttcggccagctcctcaggacaggcttgcgcgtcgatatcatcatcgctaaccaccttctcaagggcttttgtgaagcgaagcggacagacgaggctttggacatccttctccacagaacgcctgagttgggctgtgtgcccgatgttttctcgtacagcatacttctgaagagcctctgcgaccaaggaaagagtggccaggcagatgatttgctacggatgatgtctgaagggggagctgtctgctcgcccgacgtggttgcctacaatacagtaatcgacggcttctttaaggagggtgacgtaaataaagcatgtgatctattcaaagaaatggtacagcggggcattccacctgattttgtgacttatagctctgtggttcatgccctgtgtaaggcaagagcaatggacaaggcagaggctttccttcgacaaatggtcaataaaggtgttctgccaaataactggacatataataacttgatatatggatactcctccacaggacagtggaaggaggcagttagggtatttaaagaaatgagaagacatagcatcttaccagatgttgttacttttaacatgttgatgggttccctttgcaagtatggaaaaatcaaggaagctagagatgtttttgacacaatggcaatgaagggccaaaatcctgatgttttctcgtacaatattatgctcaacgggtacgctactaaaggatgtctagttgatatgacagatctcttcgatttgatgctaggtgacggtattgcacctgtcatttgtacttttaatgtgctgatcaaggcatatgcaaactgtggaatgctagataaggctatgatcatcttcaatgaaatgagagaccatggagtgaaaccttatgtgttaacctatacgacagtgattgctgccctctgcagaatcggtaagatggatgatgctatggaaaaatttaatcagatgattgatcaaggagtagcacctgataaatatgcataccattgcctgattcaaggtttttgtactcatggtagtttactgaaagccaaggaattgatttcggaaataatgaataatggcatgcatcttgacattgttttattcagttcgataattaacaacctttgcaaattgggaagggtaatggatgcacaaaatatatttgacttaactgtaaatgttggtctgcatcctactgctgtggtgtatagtatgctgatggatgggtactgtcttgttggcaagatggagaatgcattaagagtatttgatgctatggtgtcagctggcattgaaccatacgatgtagtgtatggtacacttgttaatggctattgtaaaattggaaggattgatgaaggattgagtcttttcagagaaatgctgcaaaatggaataaagccttcaactattttatacaacatcataattgatgggttatttgaggccgggagaacagttcctgcaaaggtgaaattccatgaaatgacagaaagtggtatcgctatgtacatatgtacatacatcatagttcttcgtggactttttaaaaatagatgctttgatgaagcaatctttcttttcaaagaattacgtgcaatgaatgtaaagatcgatatcataactctcaataccatgatagctggaatgtttcaaaccaggagagttgaagaagctaaggatctgtttgcttctatctcgagaagtgggctggtgccttgtgttgtgacttacagtataatgatcacaaatcttataaaagaaggattggtggaagaggcagaagatatgttttcatccatgcagaatgctggctgtgagccctattctcgattgttgaatcatgtagtcagggaattactaaagaaaaatgaaatagtcagggctggagcttacctgtccaagattgacgagaggaatttctcacttgaatatttaaccacaatgttgctggtcgatctcttctcaagcaaaggaacttgtagggaacacataagatttctccctgcaaagtatcattttcttgcagaggccagtccgtga

SEQ ID NO: 9 - protein, 814 aa, zea mays
MPSCARISSAVSTAAASSSSPPPHPPRCRRLAAATARVREGTLRPEEAHDLLDELQRRGTPVLERDLNGFLAAIARAPSSAACRSGPALAVALFNRAASRAQGPRVLSPTSHTYAILMDCCTRAHRPELALAFFGQLLRTGLRVDIIIANHLLKGFCEAKRTDEALDILLHRTPELGCVPDVFSYSILLKSLCDQGKSGQADDLLRMMAEGGAVCSPDVVAYTTVIDCFFKEGDVNKACDLFKEMVQRGIPPDFVTYSSVVHALCKARAMDKAEAFLRQMVNKGVLPNNWTYNNLIYGYSSTGQWKEAVRVFKEMRRHSILPDVVTLNMLMGSLCKYGKIKEARDVFDTMAMKGQNPNVFSYNIMLNGYATKGCLVDMTDLFDLMLGDGIAPVICTFNVLIKAYANCGMLDKAMIIFNEMRDHGVKPYVVTYTTVIAALCRIGKMDDAMEKFNQMIDQGVAPDKYAFHCLIQGFCTHGSLLKAKELILEIMNNGMRLDIVFFSSIINNLCKLGRVMEAQNIFDLTVNVGLHPTAVVYSMLMDGYCLVGKMEKALRVFDAMVSAGIEPDDVVYGTLVNGYCKIGRIDEGLSLFREMLQKGIKPSTILYNIIIDGLFQAGRTVPAKVKFHEMTESGIAMNKCTYNIVLRGLFKNRCFDEAIFLFKELRAMNVKIDIITLNTMIAGMFQTRRVEEAKDLFASISRSGLVPCVVTYSIMITNLIKEGLVEEAEDMFSSMQNAGCEPDSRLLNHVVRELLKKNEIVRAGAYLSKIDERNFSLEHLTTMLLVDLFSSKGTCREHIRFLPAKYHFLAEASP

SEQ ID NO: 10 - DNA, 2445 bp, zea mays
atgccgtcatgtgcccgcatctcctccgccgtctccaccgccgccgcatcctcctcctcgccgccgccgcatcctcctcgctgccgccgcctcgccgccgccacggcgcgcgtgcgggaggggacgctccgccctgaggaagcacacgacctgctcgacgagttgcagcgtcgaggcacgcccgttctcgagcgcgatctgaacggcttcctcgcggcgatcgcgcgtgcgccgtcctccgccgcctgcaggagtggccctgccctcgccgtcgcgctcttcaaccgcgcggcgtctcgggctcaaggaccgcgggtgctgtcccccacatcccacacctacgccatcctcatggactgctgcacccgcgcgcaccgcccagagctagcgctggcgttcttcggccagctcctcaggacaggcttgcgcgtcgatatcatcatcgctaaccaccttctcaagggcttttgtgaagcgaagcggacagacgaggctttggacatccttctccacagaacgcctgagttgggctgtgtgcccgatgttttctcgtacagcatacttctgaagagcctctgtgaccaaggaaagagtggccaggcagatgatttgttacggatgatggctgaagggggagctgtctgctcgcccgacgtggttgcctacactacagtaatcgactgcttctttaaggagggtgacgtaaataaagcatgtgatctattcaaagaaatggtacagcggggcattccacctgattttgtgacttatagctctgtggttcatgccctgtgtaaggcaagagcaatggacaaggcagaggctttccttcgacaaatggtcaataaaggtgttctgccaaataactggacatataataacttgatatatggatactcctccacaggacagtggaaggaggcagttagggtatttaaagaaatgagaagacacagcatcttaccagatgttgttactttgaacatgttgatgggttccctttgcaagtatggaaaaatcaaggaagctagagatgtttttgacacaatggcaatgaagggccaaaatcctaatgttttctcctacaatattatgctcaacgggtacgctactaaaggatgtctagttgatatgacagatctcttcgatttgatgctaggtgacggtattgcacctgtcatttgtacttttaatgtgctgatcaaggcatatgcaaactgtggaatgctagataaggctatgatcatcttcaatgaaatgagagaccatggagtgaaaccttatgtggtaacctatacgacagtgattgctgccctctgcagaatcggtaagatggatgatgctatggaaaaatttaatcagatgattgatcaaggagtagcacctgataaatatgcattccattgcctgattcaaggtttttgtactcatggtagtttactgaaagccaaggaattgattttggaaataatgaataatggcatgcgtcttgatattgttttcttcagttcgataattaacaacctttgcaaactgggaagggtaatggaggcacaaaatatatttgacttaactgtaaatgttggtctgcatcctactgctgtggtgtatagtatgcttatggatgggtactgtcttgttggcaagatggagaaagcattaagagtatttgatgctatggtgtcagctggcattgaaccagacgatgtagtgtatggtacacttgttaatggctattgtaaaattggaaggattgatgaaggattgagtcttttcagagaaatgctgcaaaagggaataaagccttcaactattttatacaacatcataattgatgggttatttcaggccgggagaacagttcctgcaaaggtgaaattccatgaaatgacagaaagtggtatcgctatgaacaaatgtacatacaacatagttcttcgtggactttttaaaaatagatgctttgatgaagcaatctttcttttcaaagaattacgtgcaatgaatgtaaagatcgatatcataactctcaataccatgatagctggaatgtttcaaaccaggagagttgaagaagctaaggatctgtttgcttctatctcgagaagtgggctggtgccttgtgttgtgacttacagtataatgatcacaaatcttataaaagaaggattggtggaagaggcagaagatatgttttcatccatgcagaatgctggctgtgagcccgattctcgattgctgaatcatgtagtcagggaattactaaagaaaaatgaaatagtcagggctggagcttacctgtccaagattgacgagaggaatttctcacttgaacatttaaccacaatgttgctggtcgatctcttctcaagcaaaggaacttgtagggaacacataagatttctccctgcaaagtatcattttcttgcagaggccagtccgtga

SEQ ID NO: 11 - protein, 615 aa, zea mays
MPSCARISSAVSTAAASSSSPPPHPPRCRRLAAATARVREGTLRPEEAHDLLDELQRRGTPVLERDLNGFLAAIARAPSSAACRSGPALAVALFNRAASRAQGPRVLSPTSHTYAILMDCCTRAHRPELALAFFGQLLRTGLRVDIIIANHLLKGFCEAKRTDEALDILLHRTPELGCVPDVFSYSILLKSLCDQGKSGQADDLLRMMSEGGAVCSPDVVAYNTVIDGFFKEGDVNKACDLFKEMVQRGIPPDFVTYSSVVHALCKARAMDKAEAFLRQMVNKGVLPNNWTYNNLIYGYSSTGQWKEAVRVFKEMRRHSILPDVVTFNMLMGSLCKYGKIKEARDVFDTMAMKGQNPDVFSYNIMLNGYATKGCLVDMTDLFDLMLGDGIAPVICTFNVLIKAYANCGMLDKAMIIFNEMRDHGVKPYVLTYTTVIAALCRIGKMDDAMEKFNQMIDQGVAPDKYAYHCLIQGFCTHGSLLKAKELISEIMNNGMHLDIVLFSSIINNLCKLGRVMDAQNIFDLTVNVGLHPTAVVYSMLMDGYCLVGKMENALRVFDAMVSAGIEPYDVVYGTLVNGYCKIGRIDEGLSLFREMLQKGIKPSTILYNIIIDGLF

SEQ ID NO: 12 - DNA, 1848 bp, zea mays
atgccgtcatgtgcccgcatctcctccgccgtctccaccgccgccgcatcctcctcctcgccgccgccgcatcctcctcgctgccgccgcctcgccgccgccacggcgcgcgtgcgggaggggacgctccgccctgaggaagcacacgacctgctcgacgagttgcagcgtcgaggcacgcccgttctcgagcgcgatctgaacggcttcctcgcggcgatcgcgcgtgcgccgtcctccgccgcctgcaggagtggccctgccctcgccgtcgcgctcttcaaccgcgcggcgtctcgggctcaaggaccgcgggtgctgtcccccacatcccacacctacgccatcctcatggactgctgcacccgcgcgcaccgcccagagctagcgctggcgttcttcggccagctcctcaggacaggcttgcgcgtcgatatcatcatcgctaaccaccttctcaagggcttttgtgaagcgaagcggacagacgaggctttggacatccttctccacagaacgcctgagttgggctgtgtgcccgatgttttctcgtacagcatacttctgaagagcctctgcgaccaaggaaagagtggccaggcagatgatttgctacggatgatgtctgaagggggagctgtctgctcgcccgacgtggttgcctacaatacagtaatcgacggcttctttaaggagggtgacgtaaataaagcatgtgatctattcaaagaaatggtacagcggggcattccacctgattttgtgacttatagctctgtggttcatgccctgtgtaaggcaagagcaatggacaaggcagaggctttccttcgacaaatggtcaataaaggtgttctgccaaataactggacatataataacttgatatatggatactcctccacaggacagtggaaggaggcagttagggtatttaaagaaatgagaagacatagcatcttaccagatgttgttacttttaacatgttgatgggttccctttgcaagtatggaaaaatcaaggaagctagagatgtttttgacacaatggcaatgaagggccaaaatcctgatgttttctcgtacaatattatgctcaacgggtacgctactaaaggatgtctagttgatatgacagatctcttcgatttgatgctaggtgacggtattgcacctgtcatttgtacttttaatgtgctgatcaaggcatatgcaaactgtggaatgctagataaggctatgatcatcttcaatgaaatgagagaccatggagtgaaaccttatgtgctaacctatacgacagtgattgctgccctctgcagaatcggtaagatggatgatgctatggaaaaatttaatcagatgattgatcaaggagtagcacctgataaatatgcataccattgcctgattcaaggtttttgtactcatggtagtttactgaaagccaaggaattgatttcggaaataatgaataatggcatgcatcttgacattgttttattcagttcgataattaacaacctttgcaaattgggaagggtaatggatgcacaaaatatatttgacttaactgtaaatgttggtctgcatcctactgctgtggtgtatagtatgctgatggatgggtactgtcttgttggcaagatggagaatgcattaagagtatttgatgctatggtgtcagctggcattgaaccatacgatgtagtgtatggtacacttgttaatggctattgtaaaattggaaggattgatgaaggattgagtcttttcagagaaatgctgcaaaagggaataaagccttcaactattttatacaacatcataattgatgggttattttag

SEQ ID NO: 13 - DNA, 24 bp, artificial sequence
  primer sequence
gattgatcaaggagtagcacctga

SEQ ID NO: 14 - DNA, 27 bp, artificial sequence
  primer sequence
cttggctttcagtaaactaccatgagt

SEQ ID NO: 15 - DNA, 18 bp, artificial sequence
  primer sequence
cataccattgcctgattc

SEQ ID NO: 16 - DNA, 26 bp, artificial sequence
  primer sequence
ggtagtttactgaaagccaaggaatt

SEQ ID NO: 17 - DNA, 26 bp, artificial sequence
  primer sequence
ttgcaaaggttgttaattatcgaact

SEQ ID NO: 18 - DNA, 19 bp, artificial sequence
  primer sequence
atggcatgcatcttgacat

SEQ ID NO: 19 - DNA, 23 bp, artificial sequence
  primer sequence
gggtactgtcttgttggcaagat

SEQ ID NO: 20 - DNA, 20 bp, artificial sequence
  primer sequence
tggttcaatgccagctgaca

SEQ ID NO: 21 - DNA, 25 bp, artificial sequence
  primer sequence
agaatgcattaagagtatttgatgc

SEQ ID NO: 22 - DNA, 22 bp, artificial sequence
  primer sequence
ggacagtggaaggaggcagtta

SEQ ID NO: 23 - DNA, 21 bp, artificial sequence
  primer sequence
ccatacttgcaaagggaaccc

SEQ ID NO: 24 - DNA, 24 bp, artificial sequence
  primer sequence
ccagatgttgttacttttaacatg

SEQ ID NO: 25 - DNA, 25 bp, artificial sequence
  primer sequence
gaataatggcatgcgtcttgatatt

SEQ ID NO: 26 - DNA, 26 bp, artificial sequence
  primer sequence
gtaggatgcagaccaacatttacagt

SEQ ID NO: 27 - DNA, 18 bp, artificial sequence
  primer sequence
cctttgcaaattgggaag

SEQ ID NO: 28 - DNA, 27 bp, artificial sequence
  primer sequence
gtactcatggtagtttactgaaagcca

SEQ ID NO: 29 - DNA, 21 bp, artificial sequence
  primer sequence
gcatccattacccttcccaat

SEQ ID NO: 30 - DNA, 26 bp, artificial sequence
  primer sequence
atcttgacattgttttattcagttcg

SEQ ID NO: 31 - DNA, 22 bp, artificial sequence
  primer sequence
gttcctgcaaaggtgaaattcc

SEQ ID NO: 32 - DNA, 24 bp, artificial sequence
  primer sequence
gaaagattgcttcatcaaagcatc

SEQ ID NO: 33 - DNA, 20 bp, artificial sequence
  primer sequence
ggtatcgctatgtacatatg

SEQ ID NO: 34 - DNA, 23 bp, artificial sequence
  primer sequence
ataacgtgccttggagtatttgg

SEQ ID NO: 35 - DNA, 22 bp, artificial sequence
  primer sequence
tggagtgaagcagatgatttgc

SEQ ID NO: 36 - DNA, 18 bp, artificial sequence
  primer sequence
ttgcatccatcttgttgc